European Patent Application EP 4 268 585 A1, published November 1, 2023. Title: 'Samkwang(SA)-flo3', floury endosperm rice mutant derived from 'Samkwang'. Applicant: REPUBLIC OF KOREA(MANAGEMENT : RURAL DEVELOPMENT ADMINISTRATION). The sequence listing filed with the application follows.

SEQUENCE LISTING (7 sequences)

SEQ ID NO: 1 - DNA, 7556 bp, Unknown
  Oryza sativa Japonica Group cultivar Samkwang(SA)-flo3 flo4-6 gene
atggctccggctcaatgtgctcgtgtgcagagggtgttccacttcggcaagggcaagagcgagggcaacaaggccatgaaggacctggtaaaaataatcgctgttgatacgagatgatgatgttatgaacttggaattttgattgttttttacactggttttggttggttgggggggggggggggtgtacagctgggagggaagggggcgaacttggcggagatggcgagcatcgggctgtcggtgccgccggggttcacggtgtcgacggaggcgtgccagcagtaccaggcggcggggaagacgctgccggcggggctgtgggaggagatcgtcgaggggctccagtgggtggaggagtacatggcggcgcgcctcggcgaccccgcccgccctctcctcctctccgtccgctccggcgccgccgtgcgtatcacttacttatatttactctctctctctcttcctctctgccacgccggcgatgtgacagatcgattgatctccgttgctgatcgatccgtgcgtgcgtgtgtgtgcaggtgtcgatgccggggatgatggacacggtgctgaacctggggctgaacgacgaggtggcggcgggactggcggccaagagcggcgaccgcttcgcgtacgactcctaccgccgtttcctcgacatgttcggcaacgtggtacgtactcctcatcagatcacactcgcccggctcgctgactcggcagctagctgcctagctcgtcggagctcacgagcttaattttactttttctctgctactttcgtgtgcgtcaacactgccacggctgcatcgacgtggtgggtaagttatttatgctgcgtcagcgacgcgacggtggtggctgcggatgcgcatacttttgtgcgttgggtggggcccggttcttccgtctcatcctatgtggggggaatttgtccgcactagagtcactccaacttcccaaagcttattgttcttttgtggctctattttactattagaaaatagggaataattttagtagtatttgactttagaaaagttacaaggagaatattttagtattgtgtcaagaaaaaaaaggaaaaaaaaacaagagatagtatgtccctctcgatcgtatatgcgattatgtgctagcaagggattaacatggaacttgctgtcaatatttgatctcctcgtacaaagaatacaagatgttttcttaggagacctgtacggcactattgccgtattttgaccatagttctttaattttattggaaaggatgactggtgaaggcgatgggtggttagcagtacaatttgacactccttactagctcagctcacatatactcctatttcatgtaataattaaattaatcagtacagggtcctccaacatagtacctgataacatctgcaatatggaaatatctgtcttcctagaagttcaaagacaagttggttgctactccagtcatacaaccaattacttttttttcacctatattcatcaaagcttattttttttggaaaaaatgttcttaattttattcttttttagcaaatttaatttagagtaaaaaacagtaagttttattatatttttcaagcgcaccgttcaccacaccggtctcggcggtctgcacaacttttgccctttgcttggggtgcgcaaccggtcggtcggtcaccttgcaccggaccggaccggtccggtcgctggagtcgaagtggttcgaactccactgcgtcccgagccctcgaccacctccctcctcctaccaatcccagccatggttcgactcatcacaagcgccgccgcggcggcggcggcggcggcgacggcggcgcggaggagagcgccctgcggaccgcgcctgagcccatcatggatgctagacctataccagcttcgattgccttggccgcgattcgctggtaagataaggccagagggtttcggtaggatgtcgcaaggatgagccgcagaatcgtgaatttgtgatgggtgttagttgttactcaatagaggggaattttgcctttattcagcccaaaaattggttacaggtcatgaatgcttcctggttcttgaatgctacagagatcagttcttagaatttttttctctctcttttccaggtcatggacattcctcatgcactgttcgaggagaagctcgaagccatgaaagcagtcaaggggctgcacaacgacactgacctgactgccactgacctcaaagaactagtggcacagtacaaggatgtctatgttgaagctaagggagagccatttccctctggtatgcccataaagtttcactcttcgtgatatctgaaattaattagtgttttgatgaaactgagccttttcttttggcgtctgaatgctaatgtactgtgttgtttgcttgccatagatcccaagaagcaactgcagctggccgtgttggccgtgttcaactcatgggatagcccaagagcaatcaagtacagaagcataaacaagatcactgggctgaagggcactgctgtaaacgtgcagaccatggtgtttggaaacatggggaacacctctggcacgggtgtgctcttcactaggaacccaagcactggagagaagaagctttacggcgaattccttgtgaatgctcaggtatggctcacaccctgttgctcctatttgcatctagctgctaactgttgcacacctgtggtttgtgtgtatgaatcaatgtatgagcaatatgtttcctgctgatcgtattgggttatgcaagcggcgataattcatatatacccgaacgatttcttataatgcaatattatttcttctgcagggtgaagatgtggttgctggaatcagaactccagaggatcttgatgctatgagggaccacatgccggagccttatgaagagctcgttgagaactgcaaaattttggagagtcactataaagaaatgatggtacaatattctaatttgctttatgcatcaataccttattagataatgggattaaggcagttctagaggcataagtgtcctacttttccctcaaactgaaacttaaaaggaagcacgatcgtctgatcatatactcgagcattgtcttggtgatatctcattacctccaatagcttgcacacagaaataagtgatttgaaacgtcttgatcatgctcttggtttagcaactaggtaatgtgcctccattatttttttttgggagactaacttaattttcatgtataatgcaggatattgaatttactgttcaggaaaataggctttggatgcttcagtgcagaacaggaaagcgcacaggaaaagatgctgtaaagattgctgtagacatggttaacgagggccttgttgagcgccgcacagcacttaagatggtagaaccaggtcacctggatcagcttcttcatcctcaggtattgtataactaagaggctctaatggtctataaactcatgcaccacataaatggacacgtacaatttcataatacctctgttatcccaaaatgccgtgttgctcttttagaacaattttgttgggttggtgtattgatgtcatagaagttaccacatcgattgcgtgcttagaataaatcagttaatacttaatagtaagctagaataatcaaagattaaatgtgtgtttgcgatctattagtgaaatttgatacgcatgtctgctttaattctgaacatcaaaatctttatgttatatttttccacaaaataggtagagtgtttgttacttgaactctgagcattttgaattatttggaatgagttttagcaaacaacagagattatctcattacgtcttgtgtagtaaagtataatactattatcataactaacaaatatcaaacataatcacacaagtattgatgttggtaactgttgttttaaaattttgttgcctgctagtttctgcacaggtcttggacattgcgtacttgagtttcagttcacaactaaattaatggcagttattgatatctcacttttaatcttttgttatgaaaaccagtttgagaacccatcagggtataaagacaaagttattgccacgggcttacctgcatcacctggggctgctgtgggccaaattgtattcactgccgaggatgctgaagcatggcatgcccaagggaaagatgttattctggtacgtcctgatcatctgtctttctaggacaaatttgtttgtttcgtccatgttagaatattaaacagctgcttataggaaaaaaaatagatttatcacagctttattcaagctgcacttgaaaactccacattgcatcgttgcatttggtgtatcttgacattttcctgtccattatgaatgtaaaggtgaggacagagaccagcccagaggatgttggtggcatgcatgcagctgttggaattcttacagcaagaggtggtatgacctctcacgctgctgttgttgcgcgcggatggggcaaatgttgtgtgtcaggatgctcaagcgtccgtgtaaatgatgcgtccaaggtgattatactagattcttgcaccacacaaacatttaagagttctcttatgtacaaaggctgcctttcacacatcgagtttgcaattaccattttatactgcagatagttgcttaatttgctgtgtctctacagattgtagtgattgaagacaaggcgctgcatgaaggtgagtggctatcgttgaatggatcaactggtgaagtgatcattggcaagcagccactctgcccaccagcccttagtggtgatttggaaactttcatgtcttgggtggatgaagttaggaaactcaaggtaagcaaaatatgtttcaagttgaagtcagctgaaaaagggacattagttttatttactcactaaggtcaaggctacctagttctgttgcaccagcatcaataaaaaatgcttattgtgagtatgttccatgttctaggttatggcaaatgctgatacccccgaggatgcaacaacagccagacagaatggggcagaaggaattgggctatgccggactgaacatatggtgtgtattaactttgtttgttaatgctctttttttttctcttttttgctaggatgatatgtgcctgaactttttagttgagtttaacatttagaagctagattcatggatgcaactcttctcttctagtcaatgcagataatttcatgccctcttctctttttcttctcttcatagttcttcgcttcagacgagaggattaaggctgtcaggcagatgattatggcttcaagtcttgaactgaggcagaaagcactagatcgccttttgccttatcagaggtctgactttgaaggcatcttccgtgcaatggatggtatgcgaaatttttaccataataatatatatgtcttaatgaatttagatgcactagtgtttaattgaaggaaacaaaaacagttttgctttcttaaatataagttaattgattgttctagtgtagatgcaacgttataaatttgcaaaagggatgcaatatacttttagaagattgcctatattatcttaacatattatgcatcatgtaagttaatgggcacgattctgctatgattcttcttttatggaaaggggtacattgatggatgtatgattcattcaacatagtcttaattcattgcatcttgcacacaacatgcttggtcatacaggcgtttaaaaatggttttttgttgcattccagggcttccggtaactattagactcttggatcctccacttcatgagttccttccagaaggccatgttgaggatatggtgcgtgagctatgctctgaaactggagcagctcaggatgatgtccttgcaagagtagaaaaactttccgaagtaaatccaatgcttggtttccgtgggtgcaggttggtttttgcactttgctattcagtgttgaattaggtctttccttttccagagcatttacttggttattgtcctactttatttgaggttgcagcaacaatctacatttgcatcattttcctttactaatgctgggaccactcaatttcaggcttggtatatcataccctgaattgactgaaatgcaagcccgtgccatctttgaagctgctataaccatgaccaaccagggtattcaagtctttccggagataatggttccccttgttggaactcctcaggtatgtgtttgctttcttcttttcattcatagtacctgacttgtgtaattgactgtctgtgaaggtgctgcaatttagatgataacttatatttacatgaattccaatttctagaatcatgcaagtattaaatcacgtgtgaatggaacattgacttcatccgggaaatggttcattccatttcttcatatttaccttctttgatgttctaatatatttgattacattgttcttttcggttggttttcaaacaattgacatttgagtattttgctgtgacaggaattggggcatcaagtggatgttatccgtcaaattgccaacaaggtgttcacagacatgggaaaaactattggctacaaagttggaactatgattgaaattcccagggcagctttagtggctgatgaggtaagaaacaactgatagctcccttcttttttgaaaatcttcagtatggttattgtcattcaacatgtagacagaactgtacatgcaacatggctagtaatagaatcttggatattaccctaaaggatattttgatcttgaaatagtgaatgattataaaaatattcaaagttcaaatgatgagtttatgttttctttaaacctataagctgacagtgctgtgttggctgcacatttattgacagatagcagagcaggctgagttcttctcctttggaacaaacgacctaacacagatgacatttggttacagtagggatgatgtggggaagttccttcccatctatctgtctcagggtatcctccagcatgacccctttgaggtaaatttgtacagccaaaatggcctcccttgataaacacccctatttcccaacatttacagatgtgagcaactcatctgcatattcttttcccaactctcgagtcctgacttctgatttggtgcaatctgaccaatttctatcatgtaacatacctgttgatgaatatattaggtgcttgatcagaggggagttggggagctggttaagctggctacagagagaggccgcaaagctaggcctaacttgaaggttagcctttcactggagctgaggacatcaccttgtatagaatccatggtttcttatattgaaatgtttttctttttttgtaaacaggtgggcatctgtggtgaacatggtggagagcctctgtcagtcgctttctttgcgaaggctgggctggactatgtttcttgttcgcctttcaggtcggttgagtgatgaaaatcgagaactctactcataaattcacagaacaatcactaactgttattaactctctttggcagggtcccaattgctaggctagctgcagctcaggtgctcctctga

SEQ ID NO: 2 - DNA, 23 bp, Artificial Sequence
  Flo4-6-RsaI-F
gatttgaaacgtcttgatcatgc

SEQ ID NO: 3 - DNA, 44 bp, Artificial Sequence
  Flo4-6-RsaI-R
agcatgaacttggtcaccttctgtctacagcaatctttacagta

SEQ ID NO: 4 - DNA, 23 bp, Artificial Sequence
  Flo4-6_FO
aatttgctttatgcatcaatacc

SEQ ID NO: 5 - DNA, 22 bp, Artificial Sequence
  Flo4-6_RO
ctgatttattctaagcacgcaa

SEQ ID NO: 6 - DNA, 24 bp, Artificial Sequence
  Flo4-6_FI
tgtctacagcaatctttacagaac

SEQ ID NO: 7 - DNA, 18 bp, Artificial Sequence
  Flo4-6_RI
aaagcgcacaggaaacga